European Patent Specification EP 3 365 428 B1, published September 4, 2024. Title: METHODS OF GENERATING HUMAN INNER EAR SENSORY EPITHELIA  AND SENSORY NEURONS. Applicant: Indiana University Research and Technology Corporation Koehler, Karl R. Hashino, Eri. The sequence listing filed with the application follows.

SEQUENCE LISTING (22 sequences)

SEQ ID NO: 1 - DNA, 22 bp, Artificial Sequence
  synthetic primer
cgtgaagaacattgatgatggc

SEQ ID NO: 2 - DNA, 20 bp, Artificial Sequence
  synthetic primer
gcgatcttcttcttgcccat

SEQ ID NO: 3 - DNA, 20 bp, Artificial Sequence
  synthetic primer
tactcgcccaagtcggaata

SEQ ID NO: 4 - DNA, 20 bp, Artificial Sequence
  synthetic primer
ttcttgggcttcccattcac

SEQ ID NO: 5 - DNA, 19 bp, Artificial Sequence
  synthetic primer
tttcagccatggaccgtca

SEQ ID NO: 6 - DNA, 20 bp, Artificial Sequence
  synthetic primer
gggagattgacctacagtgc

SEQ ID NO: 7 - DNA, 20 bp, Artificial Sequence
  synthetic primer
gggctctctgagaggcaggt

SEQ ID NO: 8 - DNA, 19 bp, Artificial Sequence
  synthetic primer
cctttgctctgcggttctg

SEQ ID NO: 9 - DNA, 20 bp, Artificial Sequence
  synthetic primer
tgcttccctgagacccagtt

SEQ ID NO: 10 - DNA, 25 bp, Artificial Sequence
  synthetic primer
gatcacttctttcctttgcatcaag

SEQ ID NO: 11 - DNA, 20 bp, Artificial Sequence
  synthetic primer
agtgagaggcaacctggaga

SEQ ID NO: 12 - DNA, 20 bp, Artificial Sequence
  synthetic primer
acactcggaccacatccttc

SEQ ID NO: 13 - DNA, 21 bp, Artificial Sequence
  synthetic primer
catgagtgtggatccagcttg

SEQ ID NO: 14 - DNA, 21 bp, Artificial Sequence
  synthetic primer
cctgaataagcagatccatgg

SEQ ID NO: 15 - DNA, 23 bp, Artificial Sequence
  synthetic primer
caacataaacggactcaatccca

SEQ ID NO: 16 - DNA, 22 bp, Artificial Sequence
  synthetic primer
accacctctacgaacacattgt

SEQ ID NO: 17 - DNA, 20 bp, Artificial Sequence
  synthetic primer
tcggatgaggcaagttagga

SEQ ID NO: 18 - DNA, 20 bp, Artificial Sequence
  synthetic primer
gtcactgtaatgggaatggg

SEQ ID NO: 19 - DNA, 64 bp, Artificial Sequence
  synthetic
gggaattttccccccattcccattacagtgactcggatgaggcaagttaggaaggtgacagaag

SEQ ID NO: 20 - DNA, 64 bp, Artificial Sequence
  synthetic
cccttaaaaggggggtaagggtaatgtcactgagcctactccgttcaatccttccactgtcttc

SEQ ID NO: 21 - DNA, 7354 bp, Artificial Sequence
  synthetic
tcgcgcgtttcggtgatgacggtgaaaacctctgacacatgcagctcccggagacggtcacagcttgtctgtaagcggatgccgggagcagacaagcccgtcagggcgcgtcagcgggtgttggcgggtgtcggggctggcttaactatgcggcatcagagcagattgtactgagagtgcaccatatgcggtgtgaaataccgcacagatgcgtaaggagaaaataccgcatcaggcgccattcgccattcaggctgcgcaactgttgggaagggcgatcggtgcgggcctcttcgctattacgccagctggcgaaagggggatgtgctgcaaggcgattaagttgggtaacgccagggttttcccagtcacgacgttgtaaaacgacggccagtgaattcgagctcggtacccggggatccccagccccagccgcatcatctcccgcaaccgccgccgccgccgcagccacctgcaactttgcaggcgagagagcatcccgtctacccgcctgagctgtccctcctggacagcaccgacccacgcgcctggctggctcccactttgcagggcatctgcacggcacgcgccgcccagtatttgctacattccccggagctgggtgcctcagaggccgctgcgccccgggacgaggtggacggccggggggagctggtaaggaggagcagcggcggtgccagcagcagcaagagccccgggccggtgaaagtgcgggaacagctgtgcaagctgaaaggcggggtggtggtagacgagctgggctgcagccgccaacgggccccttccagcaaacaggtgaatggggtgcagaagcagagacggctagcagccaacgccagggagcggcgcaggatgcatgggctgaaccacgccttcgaccagctgcgcaatgttatcccgtcgttcaacaacgacaagaagctgtccaaatatgagaccctgcagatggcccaaatctacatcaacgccttgtccgagctgctacaaacgcccagcggaggggaacagccaccgccgcctccagcctcctgcaaaagcgaccaccaccaccttcgcaccgcggcctcctatgaagggggcgcgggcaacgcgaccgcagctggggctcagcaggcttccggagggagccagcggccgaccccgcccgggagttgccggactcgcttctcagccccagcttctgcgggagggtactcggtgcagctggacgctctgcacttctcgactttcgaggacagcgccctgacagcgatgatggcgcaaaagaatttgtctccttctctccccgggagcatcttgcagccagtgcaggaggaaaacagcaaaacttcgcctcggtcccacagaagcgacggggaattttccccccattcccattacagtgactcggatgaggcaagtgctagcgccactaacttctccctgttgaaacaagcaggggatgtcgaagagaatcccgggccaatggtgagcaagggcgaggagctgttcaccggggtggtgcccatcctggtcgagctggacggcgacgtaaacggccacaagttcagcgtgtccggcgagggcgagggcgatgccacctacggcaagctgaccctgaagttcatctgcaccaccggcaagctgcccgtgccctggcccaccctcgtgaccaccctgacctacggcgtgcagtgcttcagccgctaccccgaccacatgaagcagcacgacttcttcaagtccgccatgcccgaaggctacgtccaggagcgcaccatcttcttcaaggacgacggcaactacaagacccgcgccgaggtgaagttcgagggcgacaccctggtgaaccgcatcgagctgaagggcatcgacttcaaggaggacggcaacatcctggggcacaagctggagtacaactacaacagccacaacgtctatatcatggccgacaagcagaagaacggcatcaaggtgaacttcaagatccgccacaacatcgaggacggcagcgtgcagctcgccgaccactaccagcagaacacccccatcggcgacggccccgtgctgctgcccgacaaccactacctgagcacccagtccgccctgagcaaagaccccaacgagaagcgcgatcacatggtcctgctggagttcgtgaccgccgccgggatcactctcggcatggacgagctgtacaagtaagaattccgatcatattcaataacccttaatataacttcgtataatgtatgctatacgaagttattaggtctgaagaggagtttacgtccagccaagcttaggatctcgacctcgaaattctaccgggtaggggaggcgcttttcccaaggcagtctggagcatgcgctttagcagccccgctgggcacttggcgctacacaagtggcctctggcctcgcacacattccacatccaccggtaggcgccaaccggctccgttctttggtggccccttcgcgccaccttctactcctcccctagtcaggaagttcccccccgccccgcagctcgcgtcgtgcaggacgtgacaaatggaagtagcacgtctcactagtctcgtgcagatggacagcaccgctgagcaatggaagcgggtaggcctttggggcagcggccaatagcagctttgctccttcgctttctgggctcagaggctgggaaggggtgggtccgggggcgggctcaggggcgggctcaggggcggggcgggcgcccgaaggtcctccggaggcccggcattctgcacgcttcaaaagcgcacgtctgccgcgctgttctcctcttcctcatctccgggcctttcgacctgcatccatctagatctcgagcagctgaagcttaccatgaccgagtacaagcccacggtgcgcctcgccacccgcgacgacgtccccagggccgtacgcaccctcgccgccgcgttcgccgactaccccgccacgcgccacaccgtcgatccggaccgccacatcgagcgggtcaccgagctgcaagaactcttcctcacgcgcgtcgggctcgacatcggcaaggtgtgggtcgcggacgacggcgccgcggtggcggtctggaccacgccggagagcgtcgaagcgggggcggtgttcgccgagatcggcccgcgcatggccgagttgagcggttcccggctggccgcgcagcaacagatggaaggcctcctggcgccgcaccggcccaaggagcccgcgtggttcctggccaccgtcggcgtctcgcccgaccaccagggcaagggtctgggcagcgccgtcgtgctccccggagtggaggcggccgagcgcgccggggtgcccgccttcctggagacctccgcgccccgcaacctccccttctacgagcggctcggcttcaccgtcaccgccgacgtcgaggtgcccgaaggaccgcgcacctggtgcatgacccgcaagcccggtgcctgacgcccgccccacgacccgcagcgcccgaccgaaaggagcgcacgaccccatgcatcgatgatatcagatccccgggatgcagaaattgatgatctattaaacaataaagatgtccactaaaatggaagtttttcctgtcatactttgttaagaagggtgagaacagagtacctacattttgaatggaaggattggagctacgggggtgggggtggggtgggattagataaatgcctgctctttactgaaggctctttactattgctttatgataatgtttcatagttggatatcataatttaaacaagcaaaaccaaattaagggccagctcattcctcccactcatgatctatagatctatagatctctcgtgggatcattgtttttctcttgattcccactttgtggttctaagtactgtggtttccaaatgtgtcagtttcatagcctgaagaacgagatcagcagcctctgttccacatacacttcattctcagtattgttttgccaagttctaattccatcagaagctggtcgagatccggaacccttaatataacttcgtataatgtatgctatacgaagttattaggtccctcgaagaggttcactaggcgcgccgaaggtgacagaagcctgaaaactgagacagaaacaaaactgccctttcccagtgcgcgggaagccccgcggttaaagatccccgcaccctttaatttttgctctgcgatggtcgttgtttagcaacgacttggcttcagatggcagctacatttgatggtttgcaaatgccgccgctgttccaaacttcctacggtccatattgtttgatgaaaactttctgttaaaattgtgtcctttccgcccaccttctgctccccctttagatagatacggtataattgtaggtacccgtatatggcatcattattctagttccctgctgccaatacgctgctaaaacgtcgcatcttctctgtcactggtttgggtttaatttattttacgccctgggcatccatccttgtgtgttgcgcactcaagtgtgggagatttagtcttccgaagttgttttccaaaatgcacaatgaaacgcaaaattagtgcttccaaagtggataacttttgactatggaattgttagaaaacaagaaactttaaggtttatatattgtataaacatacccagtatgtgcatccgatcgcgagaacgttggcgtcttttaggaaactccgcgcacgcactttatcagccgctgctgcggtggtggctccaggagaaactcaactgccaattgcagaccagtttttttttttttaaacacagccacttataattcttaagctctttgcaaatgtttgtttaaaaaatgaaaaattaaaaaaaatctagtagtgtcaaacgcatttggtcaattttattttgctttgttaatattagaaaacttatttattattgtttgctaccatttctacttatcttgattcattttttacgttttctactcgagatcattttattttaatttagcaaagccaactgcccttgtttaatgtattttgttttgcaaatgattaaaataaatgtgaaaagaagccttttgtcacttattccttgagttctagagtcgacctgcaggcatgcaagcttggcgtaatcatggtcatagctgtttcctgtgtgaaattgttatccgctcacaattccacacaacatacgagccggaagcataaagtgtaaagcctggggtgcctaatgagtgagctaactcacattaattgcgttgcgctcactgcccgctttccagtcgggaaacctgtcgtgccagctgcattaatgaatcggccaacgcgcggggagaggcggtttgcgtattgggcgctcttccgcttcctcgctcactgactcgctgcgctcggtcgttcggctgcggcgagcggtatcagctcactcaaaggcggtaatacggttatccacagaatcaggggataacgcaggaaagaacatgtgagcaaaaggccagcaaaaggccaggaaccgtaaaaaggccgcgttgctggcgtttttccataggctccgcccccctgacgagcatcacaaaaatcgacgctcaagtcagaggtggcgaaacccgacaggactataaagataccaggcgtttccccctggaagctccctcgtgcgctctcctgttccgaccctgccgcttaccggatacctgtccgcctttctcccttcgggaagcgtggcgctttctcatagctcacgctgtaggtatctcagttcggtgtaggtcgttcgctccaagctgggctgtgtgcacgaaccccccgttcagcccgaccgctgcgccttatccggtaactatcgtcttgagtccaacccggtaagacacgacttatcgccactggcagcagccactggtaacaggattagcagagcgaggtatgtaggcggtgctacagagttcttgaagtggtggcctaactacggctacactagaagaacagtatttggtatctgcgctctgctgaagccagttaccttcggaaaaagagttggtagctcttgatccggcaaacaaaccaccgctggtagcggtggtttttttgtttgcaagcagcagattacgcgcagaaaaaaaggatctcaagaagatcctttgatcttttctacggggtctgacgctcagtggaacgaaaactcacgttaagggattttggtcatgagattatcaaaaaggatcttcacctagatccttttaaattaaaaatgaagttttaaatcaatctaaagtatatatgagtaaacttggtctgacagttaccaatgcttaatcagtgaggcacctatctcagcgatctgtctatttcgttcatccatagttgcctgactccccgtcgtgtagataactacgatacgggagggcttaccatctggccccagtgctgcaatgataccgcgagacccacgctcaccggctccagatttatcagcaataaaccagccagccggaagggccgagcgcagaagtggtcctgcaactttatccgcctccatccagtctattaattgttgccgggaagctagagtaagtagttcgccagttaatagtttgcgcaacgttgttgccattgctacaggcatcgtggtgtcacgctcgtcgtttggtatggcttcattcagctccggttcccaacgatcaaggcgagttacatgatcccccatgttgtgcaaaaaagcggttagctccttcggtcctccgatcgttgtcagaagtaagttggccgcagtgttatcactcatggttatggcagcactgcataattctcttactgtcatgccatccgtaagatgcttttctgtgactggtgagtactcaaccaagtcattctgagaatagtgtatgcggcgaccgagttgctcttgcccggcgtcaatacgggataataccgcgccacatagcagaactttaaaagtgctcatcattggaaaacgttcttcggggcgaaaactctcaaggatcttaccgctgttgagatccagttcgatgtaacccactcgtgcacccaactgatcttcagcatcttttactttcaccagcgtttctgggtgagcaaaaacaggaaggcaaaatgccgcaaaaaagggaataagggcgacacggaaatgttgaatactcatactcttcctttttcaatattattgaagcatttatcagggttattgtctcatgagcggatacatatttgaatgtatttagaaaaataaacaaataggggttccgcgcacatttccccgaaaagtgccacctgacgtctaagaaaccattattatcatgacattaacctataaaaataggcgtatcacgaggccctttcgtc

SEQ ID NO: 22 - DNA, 3496 bp, Artificial Sequence
  synthetic
ctttgattggctgctcgcacgcgcctgcccgcgccctccattggctgagaagacacgcgaccggcgcgaggagggggttgggagaggagcggggggagactgagtggcgcgtgccgctttttaaaggggcgcagcgccttcagcaaccggagaagcatagttgcacgcgacctggtgtgtgatctccgagtgggtgggggagggtcgaggagggaaaaaaaaataagacgttgcagaagagacccggaaagggccttttttttggttgagctggtgtcccagtgctgcctccgatcctgagcctccgagcctttgcagtgcaatgtcccgcctgctgcatgcagaagagtgggctgaagtgaaggagttgggagaccaccatcgccagccccagccgcatcatctcccgcaaccgccgccgccgccgcagccacctgcaactttgcaggcgagagagcatcccgtctacccgcctgagctgtccctcctggacagcaccgacccacgcgcctggctggctcccactttgcagggcatctgcacggcacgcgccgcccagtatttgctacattccccggagctgggtgcctcagaggccgctgcgccccgggacgaggtggacggccggggggagctggtaaggaggagcagcggcggtgccagcagcagcaagagccccgggccggtgaaagtgcgggaacagctgtgcaagctgaaaggcggggtggtggtagacgagctgggctgcagccgccaacgggccccttccagcaaacaggtgaatggggtgcagaagcagagacggctagcagccaacgccagggagcggcgcaggatgcatgggctgaaccacgccttcgaccagctgcgcaatgttatcccgtcgttcaacaacgacaagaagctgtccaaatatgagaccctgcagatggcccaaatctacatcaacgccttgtccgagctgctacaaacgcccagcggaggggaacagccaccgccgcctccagcctcctgcaaaagcgaccaccaccaccttcgcaccgcggcctcctatgaagggggcgcgggcaacgcgaccgcagctggggctcagcaggcttccggagggagccagcggccgaccccgcccgggagttgccggactcgcttctcagccccagcttctgcgggagggtactcggtgcagctggacgctctgcacttctcgactttcgaggacagcgccctgacagcgatgatggcgcaaaagaatttgtctccttctctccccgggagcatcttgcagccagtgcaggaggaaaacagcaaaacttcgcctcggtcccacagaagcgacggggaattttccccccattcccattacagtgactcggatgaggcaagtgctagcgccactaacttctccctgttgaaacaagcaggggatgtcgaagagaatcccgggccaatggtgagcaagggcgaggagctgttcaccggggtggtgcccatcctggtcgagctggacggcgacgtaaacggccacaagttcagcgtgtccggcgagggcgagggcgatgccacctacggcaagctgaccctgaagttcatctgcaccaccggcaagctgcccgtgccctggcccaccctcgtgaccaccctgacctacggcgtgcagtgcttcagccgctaccccgaccacatgaagcagcacgacttcttcaagtccgccatgcccgaaggctacgtccaggagcgcaccatcttcttcaaggacgacggcaactacaagacccgcgccgaggtgaagttcgagggcgacaccctggtgaaccgcatcgagctgaagggcatcgacttcaaggaggacggcaacatcctggggcacaagctggagtacaactacaacagccacaacgtctatatcatggccgacaagcagaagaacggcatcaaggtgaacttcaagatccgccacaacatcgaggacggcagcgtgcagctcgccgaccactaccagcagaacacccccatcggcgacggccccgtgctgctgcccgacaaccactacctgagcacccagtccgccctgagcaaagaccccaacgagaagcgcgatcacatggtcctgctggagttcgtgaccgccgccgggatcactctcggcatggacgagctgtacaagtaagaattccgatcatattcaataacccttaatataacttcgtataatgtatgctatacgaagttattaggtccctcgaagaggttcactaggcgcgccgaaggtgacagaagcctgaaaactgagacagaaacaaaactgccctttcccagtgcgcgggaagccccgcggttaaagatccccgcaccctttaatttttgctctgcgatggtcgttgtttagcaacgacttggcttcagatggcagctacatttgatggtttgcaaatgccgccgctgttccaaacttcctacggtccatattgtttgatgaaaactttctgttaaaattgtgtcctttccgcccaccttctgctccccctttagatagatacggtataattgtaggtacccgtatatggcatcattattctagttccctgctgccaatacgctgctaaaacgtcgcatcttctctgtcactggtttgggtttaatttattttacgccctgggcatccatccttgtgtgttgcgcactcaagtgtgggagatttagtcttccgaagttgttttccaaaatgcacaatgaaacgcaaaattagtgcttccaaagtggataacttttgactatggaattgttagaaaacaagaaactttaaggtttatatattgtataaacatacccagtatgtgcatccgatcgcgagaacgttggcgtcttttaggaaactccgcgcacgcactttatcagccgctgctgcggtggtggctccaggagaaactcaactgccaattgcagaccagtttttttttttttaaacacagccacttataattcttaagctctttgcaaatgtttgtttaaaaaatgaaaaattaaaaaaaatctagtagtgtcaaacgcatttggtcaattttattttgctttgttaatattagaaaacttatttattattgtttgctaccatttctacttatcttgattcattttttacgttttctactcgagatcattttattttaatttagcaaagccaactgcccttgtttaatgtattttgttttgcaaatgattaaaataaatgtgaaaagaagccttttgtcacttattccttgagtataactactgaaaacaattttcaaatgaatgactttgaagaattgagttaagtcttctattcaatgtcatttatgcgatcttacagttttgaagaaaaatgttgtaaacttggtgccttcaggtagtatcaaaaccccttcaaagaaaagcactcaagtcaataattaaattgtgagataaaacttcttccaaatttgcagcacagttttgcctctttgatggccaggatctt